European Patent Application EP 4 289 954 A1, published December 13, 2023. Title: SGRNA TARGETING AQP1 MRNA, AND VECTOR AND USE THEREOF. Applicant: GUANGZHOU REFORGENE MEDICINE CO., LTD. The sequence listing filed with the application follows.

SEQUENCE LISTING (43 sequences)

SEQ ID NO: 1 - RNA, 25 nt, Artificial sequence
  Synthesized
gcccuccagaagagcuucuucuuga

SEQ ID NO: 2 - RNA, 23 nt, Artificial sequence
  Synthesized
ccuccagaagagcuucuucuuga

SEQ ID NO: 3 - RNA, 23 nt, Artificial sequence
  Synthesized
caggaacucggccaccacugccc

SEQ ID NO: 4 - RNA, 23 nt, Artificial sequence
  Synthesized
aagacaaagagggucguggccag

SEQ ID NO: 5 - RNA, 26 nt, Artificial sequence
  Synthesized
agggcagaaccgaugcugaugaagac

SEQ ID NO: 6 - RNA, 22 nt, Artificial sequence
  Synthesized
caggaacucggccaccacugcc

SEQ ID NO: 7 - RNA, 23 nt, Artificial sequence
  Synthesized
auuugaagcccagggcagaaccg

SEQ ID NO: 8 - RNA, 24 nt, Artificial sequence
  Synthesized
ugguuguuccccaccggguauuug

SEQ ID NO: 9 - RNA, 24 nt, Artificial sequence
  Synthesized
ccgucugguuguuccccaccgggu

SEQ ID NO: 10 - RNA, 23 nt, Artificial sequence
  Synthesized
ccgccgucugguuguuccccacc

SEQ ID NO: 11 - RNA, 30 nt, Artificial sequence
  Synthesized
gcgccagcguggcgaugcucagcccgaagg

SEQ ID NO: 12 - RNA, 30 nt, Artificial sequence
  Synthesized
gccagcgacaccuucacguuguccuggacc

SEQ ID NO: 13 - RNA, 23 nt, Artificial sequence
  Synthesized
aagaugcugaucuggcagcugag

SEQ ID NO: 14 - RNA, 23 nt, Artificial sequence
  Synthesized
augauguacaugagggcacggaa

SEQ ID NO: 15 - RNA, 23 nt, Artificial sequence
  Synthesized
cgaguucacaccaucagccaggu

SEQ ID NO: 16 - RNA, 23 nt, Artificial sequence
  Synthesized
gcccaggcccuggcccgaguuca

SEQ ID NO: 17 - RNA, 23 nt, Artificial sequence
  Synthesized
ucccgaugaucucgaugcccagg

SEQ ID NO: 18 - RNA, 23 nt, Artificial sequence
  Synthesized
gccaguguagucaauagccagga

SEQ ID NO: 19 - RNA, 23 nt, Artificial sequence
  Synthesized
aucccacagccaguguagucaau

SEQ ID NO: 20 - RNA, 23 nt, Artificial sequence
  Synthesized
cugaaguugugugugaucaccgc

SEQ ID NO: 21 - RNA, 23 nt, Artificial sequence
  Synthesized
cccacccagaaaauccagugguu

SEQ ID NO: 22 - RNA, 23 nt, Artificial sequence
  Synthesized
cccagaaaauccagugguugcug

SEQ ID NO: 23 - RNA, 23 nt, Artificial sequence
  Synthesized
aagucguagaugaguacagccag

SEQ ID NO: 24 - RNA, 26 nt, Artificial sequence
  Synthesized
cugcugcguggggccaggaugaaguc

SEQ ID NO: 25 - RNA, 26 nt, Artificial sequence
  Synthesized
caccuucacgcggucugugaggucac

SEQ ID NO: 26 - RNA, 29 nt, Artificial sequence
  Synthesized
gcauccaggucauacuccuccaccuggcc

SEQ ID NO: 27 - RNA, 23 nt, Artificial sequence
  Synthesized
gucauacuccuccaccuggccgc

SEQ ID NO: 28 - RNA, 20 nt, Artificial sequence
  Synthesized
gucauacuccuccaccuggc

SEQ ID NO: 29 - RNA, 23 nt, Artificial sequence
  Synthesized
gcauccaggucauacuccuccac

SEQ ID NO: 30 - RNA, 30 nt, Artificial sequence
  Synthesized
cuucaucuccacccuggaguugaugucguc

SEQ ID NO: 31 - RNA, 24 nt, Artificial sequence
  Synthesized
uuugggcuucaucuccacccugga

SEQ ID NO: 32 - RNA, 36 nt, Artificial sequence
  Synthesized
caaguaaaccccuaccaacuggucgggguuugaaac

SEQ ID NO: 33 - DNA, 7102 bp, Artificial sequence
  Synthesized
cctgcaggcagctgcgcgctcgctcgctcactgaggccgcccgggcgtcgggcgacctttggtcgcccggcctcagtgagcgagcgagcgcgcagagagggagtggccaactccatcactaggggttcctgcggcctctagactcgaggcgttgacattgattattgactagttattaatagtaatcaattacggggtcattagttcatagcccatatatggagttccgcgttacataacttacggtaaatggcccgcctggctgaccgcccaacgacccccgcccattgacgtcaataatgacgtatgttcccatagtaacgccaatagggactttccattgacgtcaatgggtggagtatttacggtaaactgcccacttggcagtacatcaagtgtatcatatgccaagtacgccccctattgacgtcaatgacggtaaatggcccgcctggcattatgcccagtacatgaccttatgggactttcctacttggcagtacatctacgtattagtcatcgctattaccatggtgatgcggttttggcagtacatcaatgggcgtggatagcggtttgactcacggggatttccaagtctccaccccattgacgtcaatgggagtttgttttggcaccaaaatcaacgggactttccaaaatgtcgtaacaactccgccccattgacgcaaatgggcggtaggcgtgtacggtgggaggtctatataagcagagctctctggctaactaccggtgccaccatgagccccaagaagaagagaaaggtggaggccagcatcgaaaaaaaaaagtccttcgccaagggcatgggcgtgaagtccacactcgtgtccggctccaaagtgtacatgacaaccttcgccgaaggcagcgacgccaggctggaaaagatcgtggagggcgacagcatcaggagcgtgaatgagggcgaggccttcagcgctgaaatggccgataaaaacgccggctataagatcggcaacgccaaattcagccatcctaagggctacgccgtggtggctaacaaccctctgtatacaggacccgtccagcaggatatgctcggcctgaaggaaactctggaaaagaggtacttcggcgagagcgctgatggcaatgacaatatttgtatccaggtgatccataacatcctggacattgaaaaaatcctcgccgaatacattaccaacgccgcctacgccgtcaacaatatctccggcctggataaggacattattggattcggcaagttctccacagtgtatacctacgacgaattcaaagaccccgagcaccatagggccgctttcaacaataacgataagctcatcaacgccatcaaggcccagtatgacgagttcgacaacttcctcgataaccccagactcggctatttcggccaggcctttttcagcaaggagggcagaaattacatcatcaattacggcaacgaatgctatgacattctggccctcctgagcggactgaggcactgggtggtccataacaacgaagaagagtccaggatctccaggacctggctctacaacctcgataagaacctcgacaacgaatacatctccaccctcaactacctctacgacaggatcaccaatgagctgaccaactccttctccaagaactccgccgccaacgtgaactatattgccgaaactctgggaatcaaccctgccgaattcgccgaacaatatttcagattcagcattatgaaagagcagaaaaacctcggattcaatatcaccaagctcagggaagtgatgctggacaggaaggatatgtccgagatcaggaaaaatcataaggtgttcgactccatcaggaccaaggtctacaccatgatggactttgtgatttataggtattacatcgaagaggatgccaaggtggctgccgccaataagtccctccccgataatgagaagtccctgagcgagaaggatatctttgtgattaacctgaggggctccttcaacgacgaccagaaggatgccctctactacgatgaagctaatagaatttggagaaagctcgaaaatatcatgcacaacatcaaggaatttaggggaaacaagacaagagagtataagaagaaggacgcccctagactgcccagaatcctgcccgctggccgtgatgtttccgccttcagcaaactcatgtatgccctgaccatgttcctggatggcaaggagatcaacgacctcctgaccaccctgattaataaattcgataacatccagagcttcctgaaggtgatgcctctcatcggagtcaacgctaagttcgtggaggaatacgcctttttcaaagactccgccaagatcgccgatgagctgaggctgatcaagtccttcgctagaatgggagaacctattgccgatgccaggagggccatgtatatcgacgccatccgtattttaggaaccaacctgtcctatgatgagctcaaggccctcgccgacaccttttccctggacgagaacggaaacaagctcaagaaaggcaagcacggcatgagaaatttcattattaataacgtgatcagcaataaaaggttccactacctgatcagatacggtgatcctgcccacctccatgagatcgccaaaaacgaggccgtggtgaagttcgtgctcggcaggatcgctgacatccagaaaaaacagggccagaacggcaagaaccagatcgacaggtactacgaaacttgtatcggaaaggataagggcaagagcgtgagcgaaaaggtggacgctctcacaaagatcatcaccggaatgaactacgaccaattcgacaagaaaaggagcgtcattgaggacaccggcagggaaaacgccgagagggagaagtttaaaaagatcatcagcctgtacctcaccgtgatctaccacatcctcaagaatattgtcaatatcaacgccaggtacgtcatcggattccattgcgtcgagcgtgatgctcaactgtacaaggagaaaggctacgacatcaatctcaagaaactggaagagaagggattcagctccgtcaccaagctctgcgctggcattgatgaaactgcccccgataagagaaaggacgtggaaaaggagatggctgaaagagccaaggagagcattgacagcctcgagagcgccaaccccaagctgtatgccaattacatcaaatacagcgacgagaagaaagccgaggagttcaccaggcagattaacagggagaaggccaaaaccgccctgaacgcctacctgaggaacaccaagtggaatgtgatcatcagggaggacctcctgagaattgacaacaagacatgtaccctgttcagaaacaaggccgtccacctggaagtggccaggtatgtccacgcctatatcaacgacattgccgaggtcaattcctacttccaactgtaccattacatcatgcagagaattatcatgaatgagaggtacgagaaaagcagcggaaaggtgtccgagtacttcgacgctgtgaatgacgagaagaagtacaacgataggctcctgaaactgctgtgtgtgcctttcggctactgtatccccaggtttaagaacctgagcatcgaggccctgttcgataggaacgaggccgccaagttcgacaaggagaaaaagaaggtgtccggcaattccggatccggacctaagaaaaagaggaaggtggcggccgcttacccatacgatgttccagattacgcttgaggtaccctagagctcgctgatcagcctcgactgtgccttctagttgccagccatctgttgtttgcccctcccccgtgccttccttgaccctggaaggtgccactcccactgtcctttcctaataaaatgaggaaattgcatcgcattgtctgagtaggtgtcattctattctggggggtggggtggggcaggacagcaagggggaggattgggaagagaatagcaggcatgctggggagagggcctatttcccatgattccttcatatttgcatatacgatacaaggctgttagagagataattggaattaatttgactgtaaacacaaagatattagtacaaaatacgtgacgtagaaagtaataatttcttgggtagtttgcagttttaaaattatgttttaaaatggactatcatatgcttaccgtaacttgaaagtatttcgatttcttggctttatatatcttgtggaaaggacgaaacaccgcaagtaaacccctaccaactggtcggggtttgaaacgggtcttcgagaagacctcaagtaaacccctaccaactggtcggggtttgaaactttttttcccgggaatggccgcaggaacccctagtgatggagttggccactccctctctgcgcgctcgctcgctcactgaggccgggcgaccaaaggtcgcccgacgcccgggctttgcccgggcggcctcagtgagcgagcgagcgcgcagctgcctgcaggggcgcctgatgcggtattttctccttacgcatctgtgcggtatttcacaccgcatacgtcaaagcaaccatagtacgcgccctgtagcggcgcattaagcgcggcgggtgtggtggttacgcgcagcgtgaccgctacacttgccagcgccctagcgcccgctcctttcgctttcttcccttcctttctcgccacgttcgccggctttccccgtcaagctctaaatcgggggctccctttagggttccgatttagtgctttacggcacctcgaccccaaaaaacttgatttgggtgatggttcacgtagtgggccatcgccctgatagacggtttttcgccctttgacgttggagtccacgttctttaatagtggactcttgttccaaactggaacaacactcaaccctatctcgggctattcttttgatttataagggattttgccgatttcggcctattggttaaaaaatgagctgatttaacaaaaatttaacgcgaattttaacaaaatattaacgtttacaattttatggtgcactctcagtacaatctgctctgatgccgcatagttaagccagccccgacacccgccaacacccgctgacgcgccctgacgggcttgtctgctcccggcatccgcttacagacaagctgtgaccgtctccgggagctgcatgtgtcagaggttttcaccgtcatcaccgaaacgcgcgagacgaaagggcctcgtgatacgcctatttttataggttaatgtcatgataataatggtttcttagacgtcaggtggcacttttcggggaaatgtgcgcggaacccctatttgtttatttttctaaatacattcaaatatgtatccgctcatgagacaataaccctgataaatgcttcaataatattgaaaaaggaagagtatgagtattcaacatttccgtgtcgcccttattcccttttttgcggcattttgccttcctgtttttgctcacccagaaacgctggtgaaagtaaaagatgctgaagatcagttgggtgcacgagtgggttacatcgaactggatctcaacagcggtaagatccttgagagttttcgccccgaagaacgttttccaatgatgagcacttttaaagttctgctatgtggcgcggtattatcccgtattgacgccgggcaagagcaactcggtcgccgcatacactattctcagaatgacttggttgagtactcaccagtcacagaaaagcatcttacggatggcatgacagtaagagaattatgcagtgctgccataaccatgagtgataacactgcggccaacttacttctgacaacgatcggaggaccgaaggagctaaccgcttttttgcacaacatgggggatcatgtaactcgccttgatcgttgggaaccggagctgaatgaagccataccaaacgacgagcgtgacaccacgatgcctgtagcaatggcaacaacgttgcgcaaactattaactggcgaactacttactctagcttcccggcaacaattaatagactggatggaggcggataaagttgcaggaccacttctgcgctcggcccttccggctggctggtttattgctgataaatctggagccggtgagcgtggaagccgcggtatcattgcagcactggggccagatggtaagccctcccgtatcgtagttatctacacgacggggagtcaggcaactatggatgaacgaaatagacagatcgctgagataggtgcctcactgattaagcattggtaactgtcagaccaagtttactcatatatactttagattgatttaaaacttcatttttaatttaaaaggatctaggtgaagatcctttttgataatctcatgaccaaaatcccttaacgtgagttttcgttccactgagcgtcagaccccgtagaaaagatcaaaggatcttcttgagatcctttttttctgcgcgtaatctgctgcttgcaaacaaaaaaaccaccgctaccagcggtggtttgtttgccggatcaagagctaccaactctttttccgaaggtaactggcttcagcagagcgcagataccaaatactgtccttctagtgtagccgtagttaggccaccacttcaagaactctgtagcaccgcctacatacctcgctctgctaatcctgttaccagtggctgctgccagtggcgataagtcgtgtcttaccgggttggactcaagacgatagttaccggataaggcgcagcggtcgggctgaacggggggttcgtgcacacagcccagcttggagcgaacgacctacaccgaactgagatacctacagcgtgagctatgagaaagcgccacgcttcccgaagggagaaaggcggacaggtatccggtaagcggcagggtcggaacaggagagcgcacgagggagcttccagggggaaacgcctggtatctttatagtcctgtcgggtttcgccacctctgacttgagcgtcgatttttgtgatgctcgtcaggggggcggagcctatggaaaaacgccagcaacgcggcctttttacggttcctggccttttgctggccttttgctcacatgt

SEQ ID NO: 34 - DNA, 23 bp, Artificial sequence
  Synthesized
gggcctatttcccatgattcctt

SEQ ID NO: 35 - DNA, 20 bp, Artificial sequence
  Synthesized
gctggcaagtgtagcggtca

SEQ ID NO: 36 - DNA, 9363 bp, Artificial sequence
  Synthesized
gtcgacggatcgggagatctcccgatcccctatggtgcactctcagtacaatctgctctgatgccgcatagttaagccagtatctgctccctgcttgtgtgttggaggtcgctgagtagtgcgcgagcaaaatttaagctacaacaaggcaaggcttgaccgacaattgcatgaagaatctgcttagggttaggcgttttgcgctgcttcgcgatgtacgggccagatatacgcgttgacattgattattgactagttattaatagtaatcaattacggggtcattagttcatagcccatatatggagttccgcgttacataacttacggtaaatggcccgcctggctgaccgcccaacgacccccgcccattgacgtcaataatgacgtatgttcccatagtaacgccaatagggactttccattgacgtcaatgggtggagtatttacggtaaactgcccacttggcagtacatcaagtgtatcatatgccaagtacgccccctattgacgtcaatgacggtaaatggcccgcctggcattatgcccagtacatgaccttatgggactttcctacttggcagtacatctacgtattagtcatcgctattaccatggtgatgcggttttggcagtacatcaatgggcgtggatagcggtttgactcacggggatttccaagtctccaccccattgacgtcaatgggagtttgttttggcaccaaaatcaacgggactttccaaaatgtcgtaacaactccgccccattgacgcaaatgggcggtaggcgtgtacggtgggaggtctatagaccagatctgagcctgggagctctctggctaactagggaacccactgcttaagcctcaataaagcttgccttgagtgcttcaagtagtgtgtgcccgtctgttgtgtgactctggtaactagagatccctcagacccttttagtcagtgtggaaaatctctagcagtggcgcccgaacagggacttgaaagcgaaagggaaaccagaggagctctctcgacgcaggactcggcttgctgaagcgcgcacggcaagaggcgaggggcggcgactggtgagtacgccaaaaattttgactagcggaggctagaaggagagagatgggtgcgagagcgtcagtattaagcgggggagaattagatcgcgatgggaaaaaattcggttaaggccagggggaaagaaaaaatataaataaacatatagtatgggcaagcagggagctagaacgattcgcagttaatcctggcctgttagaaacatcagaaggctgtagacaaatactgggacagctacaaccatcccttcagacaggatcagaagaacttagatcattatataatacagtagcaaccctctattgtgtgcatcaaaggatagagataaaagacaccaaggaagctttagacaagatagaggaagagcaaaacaaaagtaagaccaccgcacagcaagcggccggccgcgctgatcttcagacctggaggaggagatatgagggacaattggagaagtgaattatataaatataaagtagtaaaaattgaaccattaggagtagcacccaccaaggcaaagagaagagtggtgcagagagaaaaaagagcagtgggaataggagctttgttccttgggttcttgggagcagcaggaagcactatgggcgcagcgtcaatgacgctgacggtacaggccagacaattattgtctggtatagtgcagcagcagaacaatttgctgagggctattgaggcgcaacagcatctgttgcaactcacagtctggggcatcaagcagctccaggcaagaatcctggctgtggaaagatacctaaaggatcaacagctcctggggatttggggttgctctggaaaactcatttgcaccactgctgtgccttggaatgctagttggagtaataaatctctggaacagatttggaatcacacgacctggatggagtgggacagagaaattaacaattacacaagcttaatacactccttaattgaagaatcgcaaaaccagcaagaaaagaatgaacaagaattattggaattagataaatgggcaagtttgtggaattggtttaacataacaaattggctgtggtatataaaattattcataatgatagtaggaggcttggtaggtttaagaatagtttttgctgtactttctatagtgaatagagttaggcagggatattcaccattatcgtttcagacccacctcccaaccccgaggggacccgacaggcccgaaggaatagaagaagaaggtggagagagagacagagacagatccattcgattagtgaacggatcggcactgcgtgcgccaattctgcagacaaatggcagtattcatccacaattttaaaagaaaaggggggattggggggtacagtgcaggggaaagaatagtagacataatagcaacagacatacaaactaaagaattacaaaaacaaattacaaaaattcaaaattttcgggtttattacagggacagcagagatccagtttggttagtaccgggcccgctctagcgtcgaggagcttggcccattgcatacgttgtatccatatcataatatgtacatttatattggctcatgtccaacattaccgccatgttgacattgattattgactagttattaatagtaatcaattacggggtcattagttcatagcccatatatggagttccgcgttacataacttacggtaaatggcccgcctggctgaccgcccaacgacccccgcccattgacgtcaataatgacgtatgttcccatagtaacgccaatagggactttccattgacgtcaatgggtggagtatttacggtaaactgcccacttggcagtacatcaagtgtatcatatgccaagtacgccccctattgacgtcaatgacggtaaatggcccgcctggcattatgcccagtacatgaccttatgggactttcctacttggcagtacatctacgtattagtcatcgctattaccatggtgatgcggttttggcagtacatcaatgggcgtggatagcggtttgactcacggggatttccaagtctccaccccattgacgtcaatgggagtttgttttggcaccaaaatcaacgggactttccaaaatgtcgtaacaactccgccccattgacgcaaatgggcggtaggcgtgtacggtgggaggtctatataagcagagctcgtttagtgaaccgtcagatcgcctggagacgccatccacgctgttttgacctccatagaagacaccgggaccgatccagcctccgcggccccgaattcgccaccatggccagcgagttcaagaagaagctcttctggagggcagtggtggccgagttcctggccacgaccctctttgtcttcatcagcatcggttctgccctgggcttcaaatacccggtggggaacaaccagacggcggtccaggacaacgtgaaggtgtcgctggccttcgggctgagcatcgccacgctggcgcagagtgtgggccacatcagcggcgcccacctcaacccggctgtcacactggggctgctgctcagctgccagatcagcatcttccgtgccctcatgtacatcatcgcccagtgcgtgggggccatcgtcgccaccgccatcctctcaggcatcacctcctccctgactgggaactcgcttggccgcaatgacctggctgatggtgtgaactcgggccagggcctgggcatcgagatcatcgggaccctccagctggtgctatgcgtgctggctactaccgaccggaggcgccgtgaccttggtggctcagccccccttgccatcggcctctctgtagcccttggacacctcctggctattgactacactggctgtgggattaaccctgctcggtcctttggctccgcggtgatcacacacaacttcagcaaccactggattttctgggtggggccattcatcgggggagccctggctgtactcatctacgacttcatcctggccccacgcagcagtgacctcacagaccgcgtgaaggtgtggaccagcggccaggtggaggagtatgacctggatgccgacgacatcaactccagggtggagatgaagcccaaatacccatacgatgttccagattacgctggatccgctagcggcagtggagagggcagaggaagtctgctaacatgcggtgacgtcgaggagaatcctggcccagtgagcaagggcgaggagctgttcaccggggtggtgcccatcctggtcgagctggacggcgacgtaaacggccacaagttcagcgtgtccggcgagggcgagggcgatgccacctacggcaagctgaccctgaagttcatctgcaccaccggcaagctgcccgtgccctggcccaccctcgtgaccaccctgacctacggcgtgcagtgcttcagccgctaccccgaccacatgaagcagcacgacttcttcaagtccgccatgcccgaaggctacgtccaggagcgcaccatcttcttcaaggacgacggcaactacaagacccgcgccgaggtgaagttcgagggcgacaccctggtgaaccgcatcgagctgaagggcatcgacttcaaggaggacggcaacatcctggggcacaagctggagtacaactacaacagccacaacgtctatatcatggccgacaagcagaagaacggcatcaaggtgaacttcaagatccgccacaacatcgaggacggcagcgtgcagctcgccgaccactaccagcagaacacccccatcggcgacggccccgtgctgctgcccgacaaccactacctgagcacccagtccgccctgagcaaagaccccaacgagaagcgcgatcacatggtcctgctggagttcgtgaccgccgccgggatcactctcggcatggacgagctgtacaagtaaggatcctaggcggccgcgcatgccctgcaggtgatctatcgatcggccggcccctctccctccccccccccctaacgttactggccgaagccgcttggaataaggccggtgtgcgtttgtctatatgttattttccaccatattgccgtcttttggcaatgtgagggcccggaaacctggccctgtcttcttgacgagcattcctaggggtctttcccctctcgccaaaggaatgcaaggtctgttgaatgtcgtgaaggaagcagttcctctggaagcttcttgaagacaaacaacgtctgtagcgaccctttgcaggcagcggaaccccccacctggcgacaggtgcctctgcggccaaaagccacgtgtataagatacacctgcaaaggcggcacaaccccagtgccacgttgtgagttggatagttgtggaaagagtcaaatggctctcctcaagcgtattcaacaaggggctgaaggatgcccagaaggtaccccattgtatgggatctgatctggggcctcggtacacatgctttacatgtgtttagtcgaggttaaaaaaacgtctaggccccccgaaccacggggacgtggttttcctttgaaaaacacgatgataatatggccacaaccgggccggatatcacgcgtgatctgatcagcacgtgttgacaattaatcatcggcatagtatatcggcatagtataatacgacaaggtgaggaactaaaccatggccaagcctttgtctcaagaagaatccaccctcattgaaagagcaacggctacaatcaacagcatccccatctctgaagactacagcgtcgccagcgcagctctctctagcgacggccgcatcttcactggtgtcaatgtatatcattttactgggggaccttgtgcagaactcgtggtgctgggcactgctgctgctgcggcagctggcaacctgacttgtatcgtcgcgatcggaaatgagaacaggggcatcttgagcccctgcggacggtgccgacaggtgcttctcgatctgcatcctgggatcaaagccatagtgaaggacagtgatggacagccgacggcagttgggattcgtgaattgctgccctctggttatgtgtgggagggctaagcaatgcatacatgtgtttaaacctcgacttaattaagtcgagggtcgacggtatcgataagctcgcttcacgagatcatgtttaagggttccggttccactaggtacaattcgatatcaagcttatcgataatcaacctctggattacaaaatttgtgaaagattgactggtattcttaactatgttgctccttttacgctatgtggatacgctgctttaatgcctttgtatcatgctattgcttcccgtatggctttcattttctcctccttgtataaatcctggttgctgtctctttatgaggagttgtggcccgttgtcaggcaacgtggcgtggtgtgcactgtgtttgctgacgcaacccccactggttggggcattgccaccacctgtcagctcctttccgggactttcgctttccccctccctattgccacggcggaactcatcgccgcctgccttgcccgctgctggacaggggctcggctgttgggcactgacaattccgtggtgttgtcggggaaatcatcgtcctttccttggctgctcgcctgtgttgccacctggattctgcgcgggacgtccttctgctacgtcccttcggccctcaatccagcggaccttccttcccgcggcctgctgccggctctgcggcctcttccgcgtcttcgccttcgccctcagacgagtcggatctccctttgggccgcctccccgcatcgataccgtcgacctcgatcgagacctagaaaaacatggagcaatcacaagtagcaatacagcagctaccaatgctgattgtgcctggctagaagcacaagaggaggaggaggtgggttttccagtcacacctcaggtacctttaagaccaatgacttacaaggcagctgtagatcttagccactttttaaaagaaaaggggggactggaagggctaattcactcccaacgaagacaagatatccttgatctgtggatctaccacacacaaggctacttccctgattggcagaactacacaccagggccagggatcagatatccactgacctttggatggtgctacaagctagtaccagttgagcaagagaaggtagaagaagccaatgaaggagagaacacccgcttgttacaccctgtgagcctgcatgggatggatgacccggagagagaagtattagagtggaggtttgacagccgcctagcatttcatcacatggcccgagagctgcatccggactgtactgggtctctctggttagaccagatctgagcctgggagctctctggctaactagggaacccactgcttaagcctcaataaagcttgccttgagtgcttcaagtagtgtgtgcccgtctgttgtgtgactctggtaactagagatccctcagacccttttagtcagtgtggaaaatctctagcagcatgtgagcaaaaggccagcaaaaggccaggaaccgtaaaaaggccgcgttgctggcgtttttccataggctccgcccccctgacgagcatcacaaaaatcgacgctcaagtcagaggtggcgaaacccgacaggactataaagataccaggcgtttccccctggaagctccctcgtgcgctctcctgttccgaccctgccgcttaccggatacctgtccgcctttctcccttcgggaagcgtggcgctttctcatagctcacgctgtaggtatctcagttcggtgtaggtcgttcgctccaagctgggctgtgtgcacgaaccccccgttcagcccgaccgctgcgccttatccggtaactatcgtcttgagtccaacccggtaagacacgacttatcgccactggcagcagccactggtaacaggattagcagagcgaggtatgtaggcggtgctacagagttcttgaagtggtggcctaactacggctacactagaagaacagtatttggtatctgcgctctgctgaagccagttaccttcggaaaaagagttggtagctcttgatccggcaaacaaaccaccgctggtagcggtggtttttttgtttgcaagcagcagattacgcgcagaaaaaaaggatctcaagaagatcctttgatcttttctacggggtctgacgctcagtggaacgaaaactcacgttaagggattttggtcatgagattatcaaaaaggatcttcacctagatccttttaaattaaaaatgaagttttaaatcaatctaaagtatatatgagtaaacttggtctgacagttaccaatgcttaatcagtgaggcacctatctcagcgatctgtctatttcgttcatccatagttgcctgactccccgtcgtgtagataactacgatacgggagggcttaccatctggccccagtgctgcaatgataccgcgagacccacgctcaccggctccagatttatcagcaataaaccagccagccggaagggccgagcgcagaagtggtcctgcaactttatccgcctccatccagtctattaattgttgccgggaagctagagtaagtagttcgccagttaatagtttgcgcaacgttgttgccattgctacaggcatcgtggtgtcacgctcgtcgtttggtatggcttcattcagctccggttcccaacgatcaaggcgagttacatgatcccccatgttgtgcaaaaaagcggttagctccttcggtcctccgatcgttgtcagaagtaagttggccgcagtgttatcactcatggttatggcagcactgcataattctcttactgtcatgccatccgtaagatgcttttctgtgactggtgagtactcaaccaagtcattctgagaatagtgtatgcggcgaccgagttgctcttgcccggcgtcaatacgggataataccgcgccacatagcagaactttaaaagtgctcatcattggaaaacgttcttcggggcgaaaactctcaaggatcttaccgctgttgagatccagttcgatgtaacccactcgtgcacccaactgatcttcagcatcttttactttcaccagcgtttctgggtgagcaaaaacaggaaggcaaaatgccgcaaaaaagggaataagggcgacacggaaatgttgaatactcatactcttcctttttcaatattattgaagcatttatcagggttattgtctcatgagcggatacatatttgaatgtatttagaaaaataaacaaataggggttccgcgcacatttccccgaaaagtgccacctgac

SEQ ID NO: 37 - DNA, 20 bp, Artificial sequence
  Synthesized
ccatggggaaggtgaaggtc

SEQ ID NO: 38 - DNA, 21 bp, Artificial sequence
  Synthesized
gaaggggtcattgatggcaac

SEQ ID NO: 39 - DNA, 20 bp, Artificial sequence
  Synthesized
gctcttctggagggcagtgg

SEQ ID NO: 40 - DNA, 21 bp, Artificial sequence
  Synthesized
cagtgtgacagccgggttgag

SEQ ID NO: 41 - RNA, 21 nt, Artificial sequence
  Synthesized
acuuugggccagaguagcgau

SEQ ID NO: 42 - DNA, 4483 bp
  Synthesized
cctgcaggcagctgcgcgctcgctcgctcactgaggccgcccgggcgtcgggcgacctttggtcgcccggcctcagtgagcgagcgagcgcgcagagagggagtggccaactccatcactaggggttcctgcggcctctagactcgaggcgttgacattgattattgactagttattaatagtaatcaattacggggtcattagttcatagcccatatatggagttccgcgttacataacttacggtaaatggcccgcctggctgaccgcccaacgacccccgcccattgacgtcaataatgacgtatgttcccatagtaacgccaatagggactttccattgacgtcaatgggtggagtatttacggtaaactgcccacttggcagtacatcaagtgtatcatatgccaagtacgccccctattgacgtcaatgacggtaaatggcccgcctggcattatgcccagtacatgaccttatgggactttcctacttggcagtacatctacgtattagtcatcgctattaccatggtgatgcggttttggcagtacatcaatgggcgtggatagcggtttgactcacggggatttccaagtctccaccccattgacgtcaatgggagtttgttttggcaccaaaatcaacgggactttccaaaatgtcgtaacaactccgccccattgacgcaaatgggcggtaggcgtgtacggtgggaggtctatataagcagagctctctggctaactaccggtgccaccatggtgagcaagggcgaggagctgttcaccggggtggtgcccatcctggtcgagctggacggcgacgtaaacggccacaagttcagcgtgtccggcgagggcgagggcgatgccacctacggcaagctgaccctgaagttcatctgcaccaccggcaagctgcccgtgccctggcccaccctcgtgaccaccctgacctacggcgtgcagtgcttcagccgctaccccgaccacatgaagcagcacgacttcttcaagtccgccatgcccgaaggctacgtccaggagcgcaccatcttcttcaaggacgacggcaactacaagacccgcgccgaggtgaagttcgagggcgacaccctggtgaaccgcatcgagctgaagggcatcgacttcaaggaggacggcaacatcctggggcacaagctggagtacaactacaacagccacaacgtctatatcatggccgacaagcagaagaacggcatcaaggtgaacttcaagatccgccacaacatcgaggacggcagcgtgcagctcgccgaccactaccagcagaacacccccatcggcgacggccccgtgctgctgcccgacaaccactacctgagcacccagtccgccctgagcaaagaccccaacgagaagcgcgatcacatggtcctgctggagttcgtgaccgccgccgggatcactctcggcatggacgagctgtacaagtaaagcggccgaattcctagagctcgctgatcagcctcgactgtgccttctagttgccagccatctgttgtttgcccctcccccgtgccttccttgaccctggaaggtgccactcccactgtcctttcctaataaaatgaggaaattgcatcgcattgtctgagtaggtgtcattctattctggggggtggggtggggcaggacagcaagggggaggattgggaagagaatagcaggcatgctggggaggtacctttttgcggccgcaggaacccctagtgatggagttggccactccctctctgcgcgctcgctcgctcactgaggccgggcgaccaaaggtcgcccgacgcccgggctttgcccgggcggcctcagtgagcgagcgagcgcgcagctgcctgcaggggcgcctgatgcggtattttctccttacgcatctgtgcggtatttcacaccgcatacgtcaaagcaaccatagtacgcgccctgtagcggcgcattaagcgcggcgggtgtggtggttacgcgcagcgtgaccgctacacttgccagcgccctagcgcccgctcctttcgctttcttcccttcctttctcgccacgttcgccggctttccccgtcaagctctaaatcgggggctccctttagggttccgatttagtgctttacggcacctcgaccccaaaaaacttgatttgggtgatggttcacgtagtgggccatcgccctgatagacggtttttcgccctttgacgttggagtccacgttctttaatagtggactcttgttccaaactggaacaacactcaaccctatctcgggctattcttttgatttataagggattttgccgatttcggcctattggttaaaaaatgagctgatttaacaaaaatttaacgcgaattttaacaaaatattaacgtttacaattttatggtgcactctcagtacaatctgctctgatgccgcatagttaagccagccccgacacccgccaacacccgctgacgcgccctgacgggcttgtctgctcccggcatccgcttacagacaagctgtgaccgtctccgggagctgcatgtgtcagaggttttcaccgtcatcaccgaaacgcgcgagacgaaagggcctcgtgatacgcctatttttataggttaatgtcatgataataatggtttcttagacgtcaggtggcacttttcggggaaatgtgcgcggaacccctatttgtttatttttctaaatacattcaaatatgtatccgctcatgagacaataaccctgataaatgcttcaataatattgaaaaaggaagagtatgagtattcaacatttccgtgtcgcccttattcccttttttgcggcattttgccttcctgtttttgctcacccagaaacgctggtgaaagtaaaagatgctgaagatcagttgggtgcacgagtgggttacatcgaactggatctcaacagcggtaagatccttgagagttttcgccccgaagaacgttttccaatgatgagcacttttaaagttctgctatgtggcgcggtattatcccgtattgacgccgggcaagagcaactcggtcgccgcatacactattctcagaatgacttggttgagtactcaccagtcacagaaaagcatcttacggatggcatgacagtaagagaattatgcagtgctgccataaccatgagtgataacactgcggccaacttacttctgacaacgatcggaggaccgaaggagctaaccgcttttttgcacaacatgggggatcatgtaactcgccttgatcgttgggaaccggagctgaatgaagccataccaaacgacgagcgtgacaccacgatgcctgtagcaatggcaacaacgttgcgcaaactattaactggcgaactacttactctagcttcccggcaacaattaatagactggatggaggcggataaagttgcaggaccacttctgcgctcggcccttccggctggctggtttattgctgataaatctggagccggtgagcgtggaagccgcggtatcattgcagcactggggccagatggtaagccctcccgtatcgtagttatctacacgacggggagtcaggcaactatggatgaacgaaatagacagatcgctgagataggtgcctcactgattaagcattggtaactgtcagaccaagtttactcatatatactttagattgatttaaaacttcatttttaatttaaaaggatctaggtgaagatcctttttgataatctcatgaccaaaatcccttaacgtgagttttcgttccactgagcgtcagaccccgtagaaaagatcaaaggatcttcttgagatcctttttttctgcgcgtaatctgctgcttgcaaacaaaaaaaccaccgctaccagcggtggtttgtttgccggatcaagagctaccaactctttttccgaaggtaactggcttcagcagagcgcagataccaaatactgtccttctagtgtagccgtagttaggccaccacttcaagaactctgtagcaccgcctacatacctcgctctgctaatcctgttaccagtggctgctgccagtggcgataagtcgtgtcttaccgggttggactcaagacgatagttaccggataaggcgcagcggtcgggctgaacggggggttcgtgcacacagcccagcttggagcgaacgacctacaccgaactgagatacctacagcgtgagctatgagaaagcgccacgcttcccgaagggagaaaggcggacaggtatccggtaagcggcagggtcggaacaggagagcgcacgagggagcttccagggggaaacgcctggtatctttatagtcctgtcgggtttcgccacctctgacttgagcgtcgatttttgtgatgctcgtcaggggggcggagcctatggaaaaacgccagcaacgcggcctttttacggttcctggccttttgctggccttttgctcacatgt

SEQ ID NO: 43 - DNA, 7170 bp
  Synthesized
cctgcaggcagctgcgcgctcgctcgctcactgaggccgcccgggcgtcgggcgacctttggtcgcccggcctcagtgagcgagcgagcgcgcagagagggagtggccaactccatcactaggggttcctgcggcctctagactcgaggcgttgacattgattattgactagttattaatagtaatcaattacggggtcattagttcatagcccatatatggagttccgcgttacataacttacggtaaatggcccgcctggctgaccgcccaacgacccccgcccattgacgtcaataatgacgtatgttcccatagtaacgccaatagggactttccattgacgtcaatgggtggagtatttacggtaaactgcccacttggcagtacatcaagtgtatcatatgccaagtacgccccctattgacgtcaatgacggtaaatggcccgcctggcattatgcccagtacatgaccttatgggactttcctacttggcagtacatctacgtattagtcatcgctattaccatggtgatgcggttttggcagtacatcaatgggcgtggatagcggtttgactcacggggatttccaagtctccaccccattgacgtcaatgggagtttgttttggcaccaaaatcaacgggactttccaaaatgtcgtaacaactccgccccattgacgcaaatgggcggtaggcgtgtacggtgggaggtctatataagcagagctctctggctaactaccggtgccaccatgagccccaagaagaagagaaaggtggaggccagcatcgaaaaaaaaaagtccttcgccaagggcatgggcgtgaagtccacactcgtgtccggctccaaagtgtacatgacaaccttcgccgaaggcagcgacgccaggctggaaaagatcgtggagggcgacagcatcaggagcgtgaatgagggcgaggccttcagcgctgaaatggccgataaaaacgccggctataagatcggcaacgccaaattcagccatcctaagggctacgccgtggtggctaacaaccctctgtatacaggacccgtccagcaggatatgctcggcctgaaggaaactctggaaaagaggtacttcggcgagagcgctgatggcaatgacaatatttgtatccaggtgatccataacatcctggacattgaaaaaatcctcgccgaatacattaccaacgccgcctacgccgtcaacaatatctccggcctggataaggacattattggattcggcaagttctccacagtgtatacctacgacgaattcaaagaccccgagcaccatagggccgctttcaacaataacgataagctcatcaacgccatcaaggcccagtatgacgagttcgacaacttcctcgataaccccagactcggctatttcggccaggcctttttcagcaaggagggcagaaattacatcatcaattacggcaacgaatgctatgacattctggccctcctgagcggactgaggcactgggtggtccataacaacgaagaagagtccaggatctccaggacctggctctacaacctcgataagaacctcgacaacgaatacatctccaccctcaactacctctacgacaggatcaccaatgagctgaccaactccttctccaagaactccgccgccaacgtgaactatattgccgaaactctgggaatcaaccctgccgaattcgccgaacaatatttcagattcagcattatgaaagagcagaaaaacctcggattcaatatcaccaagctcagggaagtgatgctggacaggaaggatatgtccgagatcaggaaaaatcataaggtgttcgactccatcaggaccaaggtctacaccatgatggactttgtgatttataggtattacatcgaagaggatgccaaggtggctgccgccaataagtccctccccgataatgagaagtccctgagcgagaaggatatctttgtgattaacctgaggggctccttcaacgacgaccagaaggatgccctctactacgatgaagctaatagaatttggagaaagctcgaaaatatcatgcacaacatcaaggaatttaggggaaacaagacaagagagtataagaagaaggacgcccctagactgcccagaatcctgcccgctggccgtgatgtttccgccttcagcaaactcatgtatgccctgaccatgttcctggatggcaaggagatcaacgacctcctgaccaccctgattaataaattcgataacatccagagcttcctgaaggtgatgcctctcatcggagtcaacgctaagttcgtggaggaatacgcctttttcaaagactccgccaagatcgccgatgagctgaggctgatcaagtccttcgctagaatgggagaacctattgccgatgccaggagggccatgtatatcgacgccatccgtattttaggaaccaacctgtcctatgatgagctcaaggccctcgccgacaccttttccctggacgagaacggaaacaagctcaagaaaggcaagcacggcatgagaaatttcattattaataacgtgatcagcaataaaaggttccactacctgatcagatacggtgatcctgcccacctccatgagatcgccaaaaacgaggccgtggtgaagttcgtgctcggcaggatcgctgacatccagaaaaaacagggccagaacggcaagaaccagatcgacaggtactacgaaacttgtatcggaaaggataagggcaagagcgtgagcgaaaaggtggacgctctcacaaagatcatcaccggaatgaactacgaccaattcgacaagaaaaggagcgtcattgaggacaccggcagggaaaacgccgagagggagaagtttaaaaagatcatcagcctgtacctcaccgtgatctaccacatcctcaagaatattgtcaatatcaacgccaggtacgtcatcggattccattgcgtcgagcgtgatgctcaactgtacaaggagaaaggctacgacatcaatctcaagaaactggaagagaagggattcagctccgtcaccaagctctgcgctggcattgatgaaactgcccccgataagagaaaggacgtggaaaaggagatggctgaaagagccaaggagagcattgacagcctcgagagcgccaaccccaagctgtatgccaattacatcaaatacagcgacgagaagaaagccgaggagttcaccaggcagattaacagggagaaggccaaaaccgccctgaacgcctacctgaggaacaccaagtggaatgtgatcatcagggaggacctcctgagaattgacaacaagacatgtaccctgttcagaaacaaggccgtccacctggaagtggccaggtatgtccacgcctatatcaacgacattgccgaggtcaattcctacttccaactgtaccattacatcatgcagagaattatcatgaatgagaggtacgagaaaagcagcggaaaggtgtccgagtacttcgacgctgtgaatgacgagaagaagtacaacgataggctcctgaaactgctgtgtgtgcctttcggctactgtatccccaggtttaagaacctgagcatcgaggccctgttcgataggaacgaggccgccaagttcgacaaggagaaaaagaaggtgtccggcaattccggatccggacctaagaaaaagaggaaggtggcggccgcttacccatacgatgttccagattacgcttgaggtaccctagagctcgctgatcagcctcgactgtgccttctagttgccagccatctgttgtttgcccctcccccgtgccttccttgaccctggaaggtgccactcccactgtcctttcctaataaaatgaggaaattgcatcgcattgtctgagtaggtgtcattctattctggggggtggggtggggcaggacagcaagggggaggattgggaagagaatagcaggcatgctggggagagggcctatttcccatgattccttcatatttgcatatacgatacaaggctgttagagagataattggaattaatttgactgtaaacacaaagatattagtacaaaatacgtgacgtagaaagtaataatttcttgggtagtttgcagttttaaaattatgttttaaaatggactatcatatgcttaccgtaacttgaaagtatttcgatttcttggctttatatatcttgtggaaaggacgaaacaccgcaagtaaacccctaccaactggtcggggtttgaaacagggcagaaccgatgctgatgaagaccaagtaaacccctaccaactggtcggggtttgaaactttgggcttcatctccaccctggacaagtaaacccctaccaactggtcggggtttgaaactttttttcccgggaatggccgcaggaacccctagtgatggagttggccactccctctctgcgcgctcgctcgctcactgaggccgggcgaccaaaggtcgcccgacgcccgggctttgcccgggcggcctcagtgagcgagcgagcgcgcagctgcctgcaggggcgcctgatgcggtattttctccttacgcatctgtgcggtatttcacaccgcatacgtcaaagcaaccatagtacgcgccctgtagcggcgcattaagcgcggcgggtgtggtggttacgcgcagcgtgaccgctacacttgccagcgccctagcgcccgctcctttcgctttcttcccttcctttctcgccacgttcgccggctttccccgtcaagctctaaatcgggggctccctttagggttccgatttagtgctttacggcacctcgaccccaaaaaacttgatttgggtgatggttcacgtagtgggccatcgccctgatagacggtttttcgccctttgacgttggagtccacgttctttaatagtggactcttgttccaaactggaacaacactcaaccctatctcgggctattcttttgatttataagggattttgccgatttcggcctattggttaaaaaatgagctgatttaacaaaaatttaacgcgaattttaacaaaatattaacgtttacaattttatggtgcactctcagtacaatctgctctgatgccgcatagttaagccagccccgacacccgccaacacccgctgacgcgccctgacgggcttgtctgctcccggcatccgcttacagacaagctgtgaccgtctccgggagctgcatgtgtcagaggttttcaccgtcatcaccgaaacgcgcgagacgaaagggcctcgtgatacgcctatttttataggttaatgtcatgataataatggtttcttagacgtcaggtggcacttttcggggaaatgtgcgcggaacccctatttgtttatttttctaaatacattcaaatatgtatccgctcatgagacaataaccctgataaatgcttcaataatattgaaaaaggaagagtatgagtattcaacatttccgtgtcgcccttattcccttttttgcggcattttgccttcctgtttttgctcacccagaaacgctggtgaaagtaaaagatgctgaagatcagttgggtgcacgagtgggttacatcgaactggatctcaacagcggtaagatccttgagagttttcgccccgaagaacgttttccaatgatgagcacttttaaagttctgctatgtggcgcggtattatcccgtattgacgccgggcaagagcaactcggtcgccgcatacactattctcagaatgacttggttgagtactcaccagtcacagaaaagcatcttacggatggcatgacagtaagagaattatgcagtgctgccataaccatgagtgataacactgcggccaacttacttctgacaacgatcggaggaccgaaggagctaaccgcttttttgcacaacatgggggatcatgtaactcgccttgatcgttgggaaccggagctgaatgaagccataccaaacgacgagcgtgacaccacgatgcctgtagcaatggcaacaacgttgcgcaaactattaactggcgaactacttactctagcttcccggcaacaattaatagactggatggaggcggataaagttgcaggaccacttctgcgctcggcccttccggctggctggtttattgctgataaatctggagccggtgagcgtggaagccgcggtatcattgcagcactggggccagatggtaagccctcccgtatcgtagttatctacacgacggggagtcaggcaactatggatgaacgaaatagacagatcgctgagataggtgcctcactgattaagcattggtaactgtcagaccaagtttactcatatatactttagattgatttaaaacttcatttttaatttaaaaggatctaggtgaagatcctttttgataatctcatgaccaaaatcccttaacgtgagttttcgttccactgagcgtcagaccccgtagaaaagatcaaaggatcttcttgagatcctttttttctgcgcgtaatctgctgcttgcaaacaaaaaaaccaccgctaccagcggtggtttgtttgccggatcaagagctaccaactctttttccgaaggtaactggcttcagcagagcgcagataccaaatactgtccttctagtgtagccgtagttaggccaccacttcaagaactctgtagcaccgcctacatacctcgctctgctaatcctgttaccagtggctgctgccagtggcgataagtcgtgtcttaccgggttggactcaagacgatagttaccggataaggcgcagcggtcgggctgaacggggggttcgtgcacacagcccagcttggagcgaacgacctacaccgaactgagatacctacagcgtgagctatgagaaagcgccacgcttcccgaagggagaaaggcggacaggtatccggtaagcggcagggtcggaacaggagagcgcacgagggagcttccagggggaaacgcctggtatctttatagtcctgtcgggtttcgccacctctgacttgagcgtcgatttttgtgatgctcgtcaggggggcggagcctatggaaaaacgccagcaacgcggcctttttacggttcctggccttttgctggccttttgctcacatgt